European Patent Application EP 4 249 597 A1, published September 27, 2023. Title: Flavone 4'-O-methyltransferase gene and use thereof. Applicant: Suntory Holdings Limited. The sequence listing filed with the application follows.

SEQUENCE LISTING (23 sequences)

SEQ ID NO: 1 - DNA, 1056 bp, Commelina communis var. hortensis
atggaagctcaagaagacaatgcatacatgcaagcattggagctccaaactggtattgacatgaacatgactctcagggctgccattgagcttggcatcctcgaaacaatcgtcggtgccggagaaggagctaagctcgccgccggcgagatctccggccatcttccgactgccaaccccgaagctcccaacatggttgacagaatgctacgcttgctagctgctcacaatatcgtaacttgtgtcgtcgagggcggcgtcgatgggcggccggagtgcaagtatggggctgctccggtgagcaagtacttcaccggagagggtgaaatgtcgttggcaaggaaggtgttacttgcaactgatatggttacgtttcaatcatggttgcatttgaaagattcagtgataaatggtggaaatgccttccatacggctttcaatatgagcctattcgataaaaataaagtggattcacgatttaacaatgtcttcaatactagtatgaagagtgtatcgcttttcgccattaataagtttatcaacacatacgatggattcagcgatatacaagtattagttgatgttggtggcggaatcggcaccgcactttatgcaattacatccaaatttcctcatatcaagggcatcaattttgatcttccacaagtgatctctactgcacaaacttcttatccagaaatggagcatgttagtggagatatgtttgcaagtgttccaaaaggggatgccattcttttaaagcatgttcttcataattgggaggatgagagttgtttgaagatactgaaaacttgttggaattctctgccttataagggtaaggtgatcattgtggaatctgtgctcccaaaagctccgggagtttcttctgcatcaaaatattttacatgtcttgatgttattatgatggctcactttggggcaaaactaaggactattgaagagtttaaggagttatgtaacaatgctggattttcttcatttaatgctacttatttccacacatatcattgtattatggagttcactaaataa

SEQ ID NO: 2 - protein, 351 aa, Commelina communis var. hortensis
MEAQEDNAYMQALELQTGIDMNMTLRAAIELGILETIVGAGEGAKLAAGEISGHLPTANPEAPNMVDRMLRLLAAHNIVTCVVEGGVDGRPECKYGAAPVSKYFTGEGEMSLARKVLLATDMVTFQSWLHLKDSVINGGNAFHTAFNMSLFDKNKVDSRFNNVFNTSMKSVSLFAINKFINTYDGFSDIQVLVDVGGGIGTALYAITSKFPHIKGINFDLPQVISTAQTSYPEMEHVSGDMFASVPKGDAILLKHVLHNWEDESCLKILKTCWNSLPYKGKVIIVESVLPKAPGVSSASKYFTCLDVIMMAHFGAKLRTIEEFKELCNNAGFSSFNATYFHTYHCIMEFTK

SEQ ID NO: 3 - DNA, 1539 bp, Torenia hybrid cultivar
atggacacagtcttaatcacactctacaccgccctgttcgtcatcaccaccaccttcctcctcctcctccgccgaaggggaccaccgtctccgcccggtcctctctccctacccataattggccacctccacctcctcggcccaagactccaccacacgttccatgaattctcactcaaatacggcccattgatccagctcaagctcggctcgatcccgtgcgtcgtggcctcgacgcccgagctcgcgagagagtttcttaagacgaacgagctcgcgttctcctctcgcaagcactctacggccatagacatcgtcacctacgactcgtcctttgctttctctccgtacggaccctactggaagtacatcaagaaactgtgtacctacgagctgctcggagcgaggaacctcggacactttcagcccattaggaatctcgaggtcaggtcctttctgcagcttctgatgcacaagagctttaagggcgagagtgtgaatgtgacagacgagctggtgaggctgacgagcaatgtgatatcccacatgatgctgagcataaggtgctcggaagatgaaggcgatgctgaggcggcgagaacagtgatacgcgaggtgacgcagatatttggggaattcgatgttacggacataatatggttttgcaagaaattcgatctgcaggggataaagaagaggtcagaggatattcagaggaggtatgatgctttgctcgagaagattattagtgatagagagagatcgaggaggcaaaatcgtgataagcatggtggcggtaacaatgaggaggccaaggattttcttgatatgttgcttgatgtgatggagagtggggacacggaggtcaaattcactagagagcatctcaaggctttgattctggatttcttcacggccggtacggacacaacagccatagccaccgagtgggccatcgccgagctcatcaacaacccgaacgtcttgaagaaggcccaagaagaaatatcccggatcatcggaaccaagcggatcgtacaagaatccgacgccccagacctaccctacctccaggccatcatcaaggagacgttccggctccacccaccgatcccgatgctctcgcgtaagtccacctccgattgcacggtcaacggctacaaaatccaagccaagagcctcttgttcgtgaacatatggtccatcggtcgaaaccctaattactgggaaagccctatggagttcaggcccgagcggttcttggagaagggacgcgagtccatcgacgtcaagggccagcactttgagctcttgccttttgggacgggccgcaggggctgtcccggtatgttgctggctatacaagaggtggtcagcatcattgggaccatggttcagtgcttcgactggaaattggcagatggttcgggcaataatgtggacatgaccgaacggtctggattgaccgctccgagagcgttcgatctggtttgccggttgtatccacgggttgacccggccacaatatcgggtgcttga

SEQ ID NO: 4 - protein, 512 aa, Torenia hybrid cultivar
MDTVLITLYTALFVITTTFLLLLRRRGPPSPPGPLSLPIIGHLHLLGPRLHHTFHEFSLKYGPLIQLKLGSIPCVVASTPELAREFLKTNELAFSSRKHSTAIDIVTYDSSFAFSPYGPYWKYIKKLCTYELLGARNLGHFQPIRNLEVRSFLQLLMHKSFKGESVNVTDELVRLTSNVISHMMLSIRCSEDEGDAEAARTVIREVTQIFGEFDVTDIIWFCKKFDLQGIKKRSEDIQRRYDALLEKIISDRERSRRQNRDKHGGGNNEEAKDFLDMLLDVMESGDTEVKFTREHLKALILDFFTAGTDTTAIATEWAIAELINNPNVLKKAQEEISRIIGTKRIVQESDAPDLPYLQAIIKETFRLHPPIPMLSRKSTSDCTVNGYKIQAKSLLFVNIWSIGRNPNYWESPMEFRPERFLEKGRESIDVKGQHFELLPFGTGRRGCPGMLLAIQEVVSIIGTMVQCFDWKLADGSGNNVDMTERSGLTAPRAFDLVCRLYPRVDPATISGA

SEQ ID NO: 5 - DNA, 1434 bp, Gentiana triflora
atgggttctttaaccaacaatgataatcttcatattttcttagtgtgtttcattggtcaaggagttgtaaatcctatgctaagacttggcaaggcctttgcttcaaagggtctattagtcactttgtctgcaccagaaattgttggcacagaaattaggaaagccaataacctcaatgatgatcaacccataaaagttggtagtgggatgatcagatttgagttctttgatgatggatgggaatctgttaatgggtctaaaccctttgatgtttgggtgtacatcaatcatcttgatcaaactgggagacaaaaactcccaattatgctcaagaaacatgaagaaacagggacccctgtttcttgtttgattctcaatcctttagttccatgggttgcagatgttgcagacagccttcaaatcccttgtgctactctttgggttcaatcttgtgccagtttttctgcttattaccattatcaccatggtctggtacctttccctactgaatctgaaccagaaattgatgtccaattaccaggtatgccattgttgaagtacgatgaagttcctgattatttgcatccaagaactccgtatcccttctttgggaccaatattctgggtcaattcaagaacttgtccaagaatttctgcatattgatggacactttctatgaactcgaacacgagattatagacaacatgtgcaagttatgtccaattaagcctattggacccttgttcaagatcccaaaagatcccagctcaaatggtattactggaaatttcatgaaggtggatgattgtaaagagtggctggacagtagaccgacgtccacggtggtgtatgtctccgtcggcagcgtcgtttacttgaaacaagagcaagttactgagatggcctatgggattttgaactctgaagtttcgttcttgtgggttctgagacctcccagtaaacgaatcggcactgagccacatgtcttgccggaagagttctgggaaaaagccggcgatagaggcaaggttgtgcaatggagccctcaagaacaagtcttggcacatccggcaaccgtaggtttcttgactcattgtggatggaactcgacgcaggaagccatatctagcggtgtgccggtgataactttccctcagtttggtgatcaagttacgaacgccaagttcttggtggaagaattcaaagtcggggtaagattgggcagaggtgaacttgagaacagaatcatcactagagacgaggttgaaagggctctgagggagatcacgagcgggcctaaggcagaagaggtgaaagagaatgcattgaaatggaagaaaaaggcggaggagaccgtcgccaagggcggctactcggaaagaaaccttgttggtttcattgaagaggttgctagaaaaactggtaccaaataa

SEQ ID NO: 6 - protein, 477 aa, Gentiana triflora
MGSLTNNDNLHIFLVCFIGQGVVNPMLRLGKAFASKGLLVTLSAPEIVGTEIRKANNLNDDQPIKVGSGMIRFEFFDDGWESVNGSKPFDVWVYINHLDQTGRQKLPIMLKKHEETGTPVSCLILNPLVPWVADVADSLQIPCATLWVQSCASFSAYYHYHHGLVPFPTESEPEIDVQLPGMPLLKYDEVPDYLHPRTPYPFFGTNILGQFKNLSKNFCILMDTFYELEHEIIDNMCKLCPIKPIGPLFKIPKDPSSNGITGNFMKVDDCKEWLDSRPTSTVVYVSVGSVVYLKQEQVTEMAYGILNSEVSFLWVLRPPSKRIGTEPHVLPEEFWEKAGDRGKVVQWSPQEQVLAHPATVGFLTHCGWNSTQEAISSGVPVITFPQFGDQVTNAKFLVEEFKVGVRLGRGELENRIITRDEVERALREITSGPKAEEVKENALKWKKKAEETVAKGGYSERNLVGFIEEVARKTGTK

SEQ ID NO: 7 - DNA, 1927 bp, Campanula medium
accaaatgagctttgtaatttgagattaatcataattgcatgctcaactaacattctgtattcatatatccatatgtattttgacctatagatattacattacaccttgaggcctttatatatagagagtgtatctacttcccttaatatcaccttttcattcaacaagtgaagccaccatgtctatagacatatccaccctcttctatgaacttgttgcagcaatttcactctacttagctacctactctttcattcgtttcctcttcaaaccctctcaccaccaccacctccctcccggcccaaccggatggccgatcatcggagcccttccactcttaggcaccatgccacatgtttccttagccgacatggccgttaaatacggtcctataatgtacctaaaacttggttcaaagggcaccgtcgtggcctcaaatccaaaagccgcccgagccttcttgaaaacccatgatgccaatttttctaaccgtccgattgatgggggccctacctacctcgcgtataatgcacaagacatggtttttgcagaatatggcccaaaatggaagcttttgcgaaagctatgtagcttgcacatgttaggcccgaaggcactcgaggattgggctcatgtcaaagtttcagaggtcggtcatatgctcaaagaaatgtacgagcaatcgagtaagtcagtgccagtgccagtggtggtgccagagatgttaacttatgccatggctaatatgattggacgaatcatactcagccgacgcccttttgttatcacgagcaaattagactcgtctgcttctgcttctgcttctgttagtgaattccaatatatggttatggagctcatgaggatggcagggttgttcaatattggtgatttcataccatatattgcatggatggatttgcaaggcattcaacgtgatatgaaggttatacagaaaaagtttgatgtcttgttgaacaaaatgatcaaggaacatacagaatccgctcatgatcgcaaagataatcctgattttcttgatattcttatggcggctacccaagaaaacacggagggaattcagcttaatcttgtaaatgttaaggcacttcttttggatttattcacggcgggcacggatacatcatcaagtgtgatcgaatgggcactagccgaaatgttgaaccatcgacagatcctaaaccgggcccacgaagaaatggaccaagtcattggcagaaacagaagactagaacaatctgacataccaaacttgccatatttccaagccatatgcaaagaaacattccgaaaacacccttccacgcccttaaacctcccaagaatctcaacagaagcatgtgaagtggacggatttcacataccaaaaaacactagactaatagtgaacatatgggcaatagggagggaccctaaagtgtgggaaaatccattagattttactccggaacgtttcttgagtgaaaaacacgcgaaaattgatccgcgaggtaatcattttgagttaatcccatttggggctggacgaaggatatgtgcaggggctagaatgggagcggcctcggtcgagtacatattaggtacattggtgcactcatttgattggaaattgcctgatggagttgtggaagttaatatggaagagagctttgggatcgcattgcaaaaaaaagtgcctctttctgctattgttactccaagattgcctccaagttcttacactgtctaggcaaatgcttatatatatgaataattgattgagttgtttagttgtatgaaagatttgagaaaataaattattaggttttgcaccattatgttgagatggttgttgttagtgttaaggaagtcgattgtagtaataataattttatttttttcgaaaaaaaaaaaaaaaaaaaaaaa

SEQ ID NO: 8 - protein, 523 aa, Campanula medium
MSIDISTLFYELVAAISLYLATYSFIRFLFKPSHHHHLPPGPTGWPIIGALPLLGTMPHVSLADMAVKYGPIMYLKLGSKGTVVASNPKAARAFLKTHDANFSNRPIDGGPTYLAYNAQDMVFAEYGPKWKLLRKLCSLHMLGPKALEDWAHVKVSEVGHMLKEMYEQSSKSVPVPVVVPEMLTYAMANMIGRIILSRRPFVITSKLDSSASASASVSEFQYMVMELMRMAGLFNIGDFIPYIAWMDLQGIQRDMKVIQKKFDVLLNKMIKEHTESAHDRKDNPDFLDILMAATQENTEGIQLNLVNVKALLLDLFTAGTDTSSSVIEWALAEMLNHRQILNRAHEEMDQVIGRNRRLEQSDIPNLPYFQAICKETFRKHPSTPLNLPRISTEACEVDGFHIPKNTRLIVNIWAIGRDPKVWENPLDFTPERFLSEKHAKIDPRGNHFELIPFGAGRRICAGARMGAASVEYILGTLVHSFDWKLPDGVVEVNMEESFGIALQKKVPLSAIVTPRLPPSSYTV

SEQ ID NO: 9 - DNA, 720 bp, Torenia hybrid cultivar
atgaaagataagttctatggcaccattttgcagagcgaagccctcgcaaagtatctgttagagacaagtgcctatccacgagaacatccgcagctcaaagaactaaggagcgcaactgtggacaagtatcaatattggagcttgatgaatgttccagctgatgaggggcagttcatttcaatgttactgaaaattatgaacgcaaaaaagacaattgaagttggagttttcacaggctactcactcctatcaactgctctggctctacctgatgatggcaaaatcgttgccattgatcctgatagagaagcttatgagactggtttgccatttatcaagaaagcaaacgtggctcataaaatccaatacatacaatctgatgccatgaaagtcatgaatgacctcattgctgccaagggagaagaagaagaggggagctttgactttgggttcgtggatgcagacaaagaaaactacataaactaccacgagaaactgttgaagctggttaaggttggagggatcataggatacgacaacactctgtggtctggaacagttgctgcatctgaagacgatgagaataatatgcaagactacttaagaggttgcagagggcatatcctcaaactaaactcctttctcgcaaacgatgatcggattgaattggctcacctctctattggagatggactcaccttgtgcaaacgtctcaaataa

SEQ ID NO: 10 - protein, 239 aa, Torenia hybrid cultivar
MKDKFYGTILQSEALAKYLLETSAYPREHPQLKELRSATVDKYQYWSLMNVPADEGQFISMLLKIMNAKKTIEVGVFTGYSLLSTALALPDDGKIVAIDPDREAYETGLPFIKKANVAHKIQYIQSDAMKVMNDLIAAKGEEEEGSFDFGFVDADKENYINYHEKLLKLVKVGGIIGYDNTLWSGTVAASEDDENNMQDYLRGCRGHILKLNSFLANDDRIELAHLSIGDGLTLCKRLK

SEQ ID NO: 11 - DNA, 58 bp, Arabidopsis thaliana
tacatcacaatcacacaaaactaacaaaagatcaaaagcaagttcttcactgttgata

SEQ ID NO: 12 - DNA, 1920 bp, Glycyrrhiza echinata
ccccaatttcctctatcataagccattccgttgattgagcttcctttccgtgaaaaaaataactaagcgatatggaacctcaactcgtagcagtgtctgtgttggtttcagcacttatctgctacttctttttccggccatatttccaccgttacggaaaaaaccttccaccatctccttttttccggcttccaataattggccacatgcacatgttaggtccccttcttcaccaatccttccacaacctctcccaccgttacggtcctctgttttcacttaactttggctctgttctctgtgtcgttgcttcaacccctcactttgccaaacaactccttcaaaccaacgaactcgcctttaactgtcgcattgaatcaaccgccgttaaaaaactcacttacgagtcttccttggccttcgcaccttacggtgattactggaggttcattaagaagctgagcatgaacgagcttttgggctctcgtagcataaacaacttccaacacctacgagcacaagagacccatcaattgttaaggcttttgtccaacagggcaagagcgtttgaggccgtgaatatcaccgaggagcttcttaagttgaccaacaacgttatttctataatgatggttggggaggcagaggaggcaagggatgtggtgcgtgatgtgacggagatatttggagagtttaatgtttcggattttatttggttgtttaagaagatggacttgcaggggtttgggaagaggattgaggatttgtttcagaggtttgatacgttggtggaaaggattattagcaagcgggagcagacgaggaaagacagaaggaggaatgggaagaagggtgagcaggggagtggtgatgggatcagagactttcttgatatcttgcttgactgtactgaggatgagaattccgagattaaaatccaaagggttcacattaaggccttgattatggatttcttcactgcagggacggataccacagcgatttcaacagagtgggcattagtggagctcgtcaagaaaccctccgtgctacaaaaagttcgtgaagagatagacaatgtcgtaggaaaagacagacttgttgaggaatctgattgtcctaatctcccatatctccaagccattcttaaagaaacattccgtttgcacccaccggttcctatggttacaagaagatgcgtggcagagtgcacggtagagaattacgtcatcccagaagactcacttctctttgtgaatgtttggtccatcggaagaaacccaaagttttgggacaacccattggagtttcgccccgaacgattcttaaaactagaaggagattccagtggagttgttgatgtgaggggaagccattttcagcttctgccatttgggtctggaaggaggatgtgccctggtgtgtccttggctatgcaagaggtgccagcactacttggtgctataatccagtgctttgatttccacgttgtgggtcccaaaggtgagattttgaagggtgatgacatagtcattaatgtggatgaaaggccaggattgacggctccaagggcacataaccttgtgtgtgttcccgttgatagaacaagtggcggtggacccctcaaaatcattgaatgttgattattcgtctcttgaatttggatctgtgtgtggctttgaataacatgtatggtgtatgtatgtatgtgttcttttctttctttctaattctgatcagtagcgtacactaggcactagccttcgttagtggcaataacttcggcaaattaacgaacatatgctgttcagagatattttttgccatgtatcgtcattctattctaggttgtttttccgttttccttattacattctatgataaatataataaattgagtaatattatagtctcttaatt

SEQ ID NO: 13 - protein, 523 aa, Glycyrrhiza echinata
MEPQLVAVSVLVSALICYFFFRPYFHRYGKNLPPSPFFRLPIIGHMHMLGPLLHQSFHNLSHRYGPLFSLNFGSVLCVVASTPHFAKQLLQTNELAFNCRIESTAVKKLTYESSLAFAPYGDYWRFIKKLSMNELLGSRSINNFQHLRAQETHQLLRLLSNRARAFEAVNITEELLKLTNNVISIMMVGEAEEARDVVRDVTEIFGEFNVSDFIWLFKKMDLQGFGKRIEDLFQRFDTLVERIISKREQTRKDRRRNGKKGEQGSGDGIRDFLDILLDCTEDENSEIKIQRVHIKALIMDFFTAGTDTTAISTEWALVELVKKPSVLQKVREEIDNVVGKDRLVEESDCPNLPYLQAILKETFRLHPPVPMVTRRCVAECTVENYVIPEDSLLFVNVWSIGRNPKFWDNPLEFRPERFLKLEGDSSGVVDVRGSHFQLLPFGSGRRMCPGVSLAMQEVPALLGAIIQCFDFHVVGPKGEILKGDDIVINVDERPGLTAPRAHNLVCVPVDRTSGGGPLKIIEC

SEQ ID NO: 14 - DNA, 990 bp, Lotus japonicus
atggcttctgcaacaaccaccccaaccaaagagatagacagagacctccctcctcttctccgagtctacaaagatggaaccgtggaacgtctcctaggctctcctgtcgttccagcaatccctcatgacccagaaacagaggtctcatcaaaagacatagtcatctcacaaacccccttaatctctgctcgtatccacctcccaaaacagagcaacccccaaaacccaaaggttccaatattgatctactaccatggtggtgcgttttgccttgaatcagctttctccttcctccaccaacgctacctcaacatcgtggcttcacgatcaaacgttgtggtggtttccgtcgagtacaggctcgcgccagagcatcctctgcctgcagcatatgaagatggttgggaagctctgaaatgggttacctctcattccaccgacaacaaacccatcaactctgagccatggttgatcgaacatggtgatttcagcagattctacatcggaggtgacacttcaggtgccaacatcgcataccatgtgggtctccgtgtcggtggtggagttgagaaattgccaggggatgtgaaaattgcaggggcgttacttgcttttcccctgttttggagttcataccctgttttggaagaacctgttgaggggtttgaacagagtttgagcaggaaggtttggaactttgtgtacccagatgcacctggtgggatcgacaaccctctgatcaatcctttggctgatggggctccaagcttgacaacgtttggaagcaacaagatgttgatctttgttgcagggaatgatgaactgagagacagaggaatctggttctatgaggctgtgaagaagagtgagtgggaaggtgatgtggaactcattcgagtggatggagaggagcattgcttccagatttaccatcctgaatctgagaattctaaagacatgatgaagcgcatagcttctttccttgtttga

SEQ ID NO: 15 - protein, 329 aa, Lotus japonicus
MASATTTPTKEIDRDLPPLLRVYKDGTVERLLGSPVVPAIPHDPETEVSSKDIVISQTPLISARIHLPKQSNPQNPKVPILIYYHGGAFCLESAFSFLHQRYLNIVASRSNVVVVSVEYRLAPEHPLPAAYEDGWEALKWVTSHSTDNKPINSEPWLIEHGDFSRFYIGGDTSGANIAYHVGLRVGGGVEKLPGDVKIAGALLAFPLFWSSYPVLEEPVEGFEQSLSRKVWNFVYPDAPGGIDNPLINPLADGAPSLTTFGSNKMLIFVAGNDELRDRGIWFYEAVKKSEWEGDVELIRVDGEEHCFQIYHPESENSKDMMKRIASFLV

SEQ ID NO: 16 - DNA, 1374 bp, Fagopyrum esculentum
atgatgggcgacttaaccacatcttttccagcaaccacactcaccacgaatgatcaacctcacgtggtggtttgctcaggagctggtatggggcatttgacaccgttccttaacttggcctctgctctttcatctgcgccgtataactgcaaggttactctgttaatcgtgattccgcttatcacagatgccgaaagtcaccacattagcagtttcttctcttcacatcccactatccacaggctagacttccacgtgaatttaccggctccaaagcccaatgtggatccgttctttctccgttacaagagcatctcagactctgcacatagacttcctgtccacttatcggccttgagtcccccgatatctgccgttttctctgacttcctcttcactcagggtctgaacactactttgcctcatcttcccaactacacgtttactacgacttctgctcggtttttcaccttgatgtcctatgttcctcacttggccaaatcgagctcatcaagtcctgtagagattcctggccttgagccgtttccaactgacaacatccctcccccttttttcaacccagagcacatctttaccagtttcaccatatccaatgccaagtacttctcgttgagcaaagggattttggtgaataccttcgactcctttgagcccgagacactctctgcattgaactcgggagacacattgtcagatctccctccggtcatccctattggcccactgaacgaactcgagcataacaaacaggaggaactcctgccatggctcgaccaacaacctgagaaatccgtcctttacgtctcttttgggaatcgaacagccatgagtagcgatcagattctcgagctaggaatgggattagagcgtagtgattgtcgctttatttgggtcgttaagacgtccaagatagacaaggacgataagagtgagctacgtaaactctttggtgaagagctctaccttaaactgtccgagaagggaaagcttgtgaaatgggtgaaccaaaccgagattctcgggcatactgctgtaggtggtttcctgtctcattgtgggtggaattcggtcatggaagcagccagaagaggtgttccgatattggcttggccacaacacggtgatcagcgggaaaatgcatgggttgttgaaaaggctggcttgggagtgtgggaaagggagtgggcaagcgggattcaggcagccattgttgagaaggtcaagatgatcatgggcaataacgaccttcgcaaaagcgctatgaaggtgggtgaagaggcaaagcgagcatgtgatgtaggtgggagttccgctaccgccttgatgaatattatcgggtcattgaagaggtaa

SEQ ID NO: 17 - protein, 457 aa, Fagopyrum esculentum
MMGDLTTSFPATTLTTNDQPHVVVCSGAGMGHLTPFLNLASALSSAPYNCKVTLLIVIPLITDAESHHISSFFSSHPTIHRLDFHVNLPAPKPNVDPFFLRYKSISDSAHRLPVHLSALSPPISAVFSDFLFTQGLNTTLPHLPNYTFTTTSARFFTLMSYVPHLAKSSSSSPVEIPGLEPFPTDNIPPPFFNPEHIFTSFTISNAKYFSLSKGILVNTFDSFEPETLSALNSGDTLSDLPPVIPIGPLNELEHNKQEELLPWLDQQPEKSVLYVSFGNRTAMSSDQILELGMGLERSDCRFIWVVKTSKIDKDDKSELRKLFGEELYLKLSEKGKLVKWVNQTEILGHTAVGGFLSHCGWNSVMEAARRGVPILAWPQHGDQRENAWVVEKAGLGVWEREWASGIQAAIVEKVKMIMGNNDLRKSAMKVGEEAKRACDVGGSSATALMNIIGSLKR

SEQ ID NO: 18 - DNA, 71 bp, Arabidopsis thaliana
acaaattcaaaatttaacacacaaacacaaacacacacaccaaaaaaaacacagaccttaaaaaaataaaa

SEQ ID NO: 19 - DNA, 1492 bp, Iris japonica
atgggttccaactctactcctgattctaccagcgaggtcaaggtgtttgactttaaagctctaatggatgacactgtagaaaagttccagaagttgatggccctaaagtgcgcaatggagctcggcattccgcatgccatcaaccgggggcaaggcaaaccaatcagcctccaacagttgatgtccgagctctcgctcccttccgccagggccccgtgcttggctcggctaatgcgcttactgacgctcatgggctgcttcgcaaagaagtcggtcgacgacgaagaagaaagatatgtatcaacaccttcgtctctccgactatgcgaagaccttaattctctttattcgtattttgcattgcatcgtgctattgcagagccatggttccacatgagctcctggctccgcggggacgcgcccactcccttccatttggcattcggaatgaacttttgggagtatgccggtcggaaccccgagttcaacaagacgttcaacaagattatgtccgacgactcgaaacaaatagtcgatgaaatggtgaagaaacatagttcagtgctcgacggggttaaatcactcgtcgacatcggtggcggcgatggcacggtggcaagggatatcgtgcgggccttccctcaggtgaagtgctacgtgtttgatcttccccatgttgtagccacggtcgatcaacaaagtgatcatgtggtggaatatattccaggaagcatgtttgaatacattccctcagctgatgcatttcttctcaagaggattttgcatgattatgaagacgaggaatgtataaagatattaaagttgtgcaaagaagcaatttcaaaacaggagggatcaggaaaaataattatacttgatgtgattgttaataaggaggatacgttcccgatgacagagtatcacacactccttgatcttcaaatgatggcaatcttagcaggtaaggaacgggaggagcaagaatggcaaaagattttcaatgaagctggtttcacgagctacaaaataataccaatgaccaaattaagtttgatcgagctcaagctttaatcatccactcagatgaccatgcatgtccttagacatttatcctctagagtcgataagtatttggttgaattctatttccgtaatcttatttatgtactagtgaataattggatgatgattcaaattaataaagatatgccaaacacctctagctcatgtgactaaggtgagaggtattttccctagctaggtgggcttgatcctctctatggtaggcaagttcgtgtggattcttatgggattgttgggtgggtggtgtgtgtgttttcaaaaaattaataaaaacatttttagggtaaatattgttgagtcagtttcgagtccatcaattatatgattgcttgattgtccatcaattatatgatttcttgattgtcattgtgtattttgaataaataggatgtttatggaaaaaaaaaaa

SEQ ID NO: 20 - protein, 356 aa, Iris japonica
MGSNSTPDSTSEVKVFDFKALMDDTVEKFQKLMALKCAMELGIPHAINRGQGKPISLQQLMSELSLPSARAPCLARLMRLLTLMGCFAKKSVDDEEERYVSTPSSLRLCEDLNSLYSYFALHRAIAEPWFHMSSWLRGDAPTPFHLAFGMNFWEYAGRNPEFNKTFNKIMSDDSKQIVDEMVKKHSSVLDGVKSLVDIGGGDGTVARDIVRAFPQVKCYVFDLPHVVATVDQQSDHVVEYIPGSMFEYIPSADAFLLKRILHDYEDEECIKILKLCKEAISKQEGSGKIIILDVIVNKEDTFPMTEYHTLLDLQMMAILAGKEREEQEWQKIFNEAGFTSYKIIPMTKLSLIELKL

SEQ ID NO: 21 - DNA, 1071 bp, Iris japonica
atggggagtaacagtactcctgattccacatcggaagtcaaggttttcgattttaaggcattgatggacgatacagttgagaagttccagaagttgatggctctcaagtgtgccatggagctgggcattccacatgccatcaatcgcggtcaagggaaaccgatttccttgcagcagttgatgagcgagttaagtctcccttcagctcgtgcaccgtgtttagccaggcttatgcgacttcttaccctgatgggatgtttcgccaagaagagcgttgacgatgaggaggagagatacgtctctacaccaagttcattgcggctttgtgaagacctgaactcgctctacagctactttgccctacatagggctattgccgaaccttggttccacatgtcgtcttggttgcgtggagatgcacctactccgtttcaccttgcattcggcatgaacttttgggagtacgcaggtagaaatcccgagttcaataagaccttcaacaagattatgtcagatgactctaagcagatcgtggatgagatggtcaagaaacactcttctgttctcgacggagtgaagagtctcgtggatataggtgggggtgatggcactgttgctagggacattgtgcgtgctttcccacaagtgaagtgctacgtctttgacttacctcacgtagtcgcaacagttgaccagcaatcagaccatgtggtagagtacattcctggtagcatgttcgaatacataccctcagcagatgcgtttcttttgaaacggatcttacacgactatgaggacgaagagtgcatcaagattctgaaactctgtaaagaagccatatctaagcaagaaggatccgggaagatcattatcctagacgttattgtgaacaaagaggacacttttcccatgaccgagtatcatacgctgttggatctccagatgatggccatacttgctgggaaagaacgcgaagagcaagagtggcaaaagatcttcaatgaggctggttttacgtcttacaagatcattccgatgaccaaactctccttgattgagttgaaactctaa

SEQ ID NO: 22 - DNA, 1443 bp, Eutrema japonicum
atggagctcgaaacttcttcatctccgaacccaattcatgtaatgctcgtgtcgtttcaaggacaaggcagcgtcagtcctcttcttcgtctcggcaagcttattgcttcaaagggaccagtcgtcaccttcgtcactacggagttttggggcaagaaaatgagacaagccaacaagatcgtcgacggtgagcttaaaccggttggttccggttatatccggtttgagtttttcgacgacggatgggcagaggatgacgcacggagaggtgatttcgatttgtacctctcacagctcgaacaagccgggaaacgacaagtgtcgaaaatcgtgaggagatacgaggaaaagaacgatcccgtctcgtgtctgatcaataacccgtttatcccatgggtcggccacgtggcggaagagttcaacattctctacgctgttctctggatccagtcttgtgcttgtttctctacttattaccattaccaaaacggctctgtttctttcccgacagaaacagagcctaagctcgatgttaagctcccttgcgctcctgtcttgaagcacgacgagatccccacctttctccatccttcttcttcgcacttcaccgcaatgcgacaagcggcccttggaatattcgagaatctgagtaagcccttctgtgttctaatcagttccttcgacgccttggaacaagaagtgatcgattatatgtcgaaactctgtccgatcaaaaccgttggaccgcttttcaaagtcgctaagacggtgatctctgatgtcagcggtgacttctgcaaaccgtcggatcaatgcctcgagtggttagactcgaggccgagatcgtccgttgtctacatttctttcgggacggttgcgtatttgaagcaagaacagatggaagagatcgctcgaggggttttgcaatcgggtttatcgttcttgtgggtgattagacctccactagaggatctaaggctcgaggctcatgtcgtgcctcgagaactgaaagaagccagtgataaaggtatagggaagattgtggattggtgtccacaagaccaagtcttggctcatccttcattggcgtgtttcgtcactcattgtgggtggaattcgacgacggaggctttgtcttcgggagttccggtggtttgttttccgcaatggggagatcaagtgaccaacgcggtttatatggttgatgttttcaagacggcagtgaggcttggccggggagcggccgaggggagggttgtgccgggggaggaagtggcggagaagcttttggaagcgacggttggggagaaagcggaggagctgagaaagaatgcattgaaatggaaagcggagtcggaagcggctgtggctcccgggggttcgtcggaaaagaatttccgggagtttatggagaagttaggggtcaaggagaacggacactag

SEQ ID NO: 23 - protein, 480 aa, Eutrema japonicum
MELETSSSPNPIHVMLVSFQGQGSVSPLLRLGKLIASKGPVVTFVTTEFWGKKMRQANKIVDGELKPVGSGYIRFEFFDDGWAEDDARRGDFDLYLSQLEQAGKRQVSKIVRRYEEKNDPVSCLINNPFIPWVGHVAEEFNILYAVLWIQSCACFSTYYHYQNGSVSFPTETEPKLDVKLPCAPVLKHDEIPTFLHPSSSHFTAMRQAALGIFENLSKPFCVLISSFDALEQEVIDYMSKLCPIKTVGPLFKVAKTVISDVSGDFCKPSDQCLEWLDSRPRSSVVYISFGTVAYLKQEQMEEIARGVLQSGLSFLWVIRPPLEDLRLEAHVVPRELKEASDKGIGKIVDWCPQDQVLAHPSLACFVTHCGWNSTTEALSSGVPVVCFPQWGDQVTNAVYMVDVFKTAVRLGRGAAEGRVVPGEEVAEKLLEATVGEKAEELRKNALKWKAESEAAVAPGGSSEKNFREFMEKLGVKENGH